European Patent Application EP 4 477 659 A1, published December 18, 2024. Title: オリゴヌクレオチドの製造方法. Applicant: SUMITOMO CHEMICAL COMPANY, LIMITED. Application JP, filed July 14, 2023. The sequence listing filed with the application follows.

SEQUENCE LISTING (10 sequences)

SEQ ID NO: 1 - RNA, 21 nt, synthetic construct
  misc_feature 1..21: note = Synthetic oligonucleotide
  modified_base join(7,17): mod_base = um
  misc_feature 20..21: note = modified base - dT
  source 1..21: mol_type = other RNA
atggaanactcttggtnacnn

SEQ ID NO: 2 - RNA, 21 nt, synthetic construct
  misc_feature 1..21: note = Synthetic oligonucleotide
  misc_feature join(2,12,14..15,19): note = modified base - um
  misc_feature join(5..6,16..17): note = modified base - cm
  misc_feature 20..21: note = modified base - dT
  source 1..21: mol_type = other RNA
gnaannaagagnannnnannn

SEQ ID NO: 3 - RNA, 36 nt, synthetic construct
  misc_feature 1..36: note = Synthetic oligonucleotide
  source 1..36: mol_type = other RNA
agagccagccttcttattgttttagagctatgctgt

SEQ ID NO: 4 - RNA, 23 nt, synthetic construct
  misc_feature 1..23: note = Synthetic oligonucleotide
  source 1..23: mol_type = other RNA
ccatgagaagtatgacaacagcc

SEQ ID NO: 5 - RNA, 25 nt, synthetic construct
  misc_feature 1..25: note = Synthetic oligonucleotide
  source 1..25: mol_type = other RNA
ggctgttgtcatacttctcatggtt

SEQ ID NO: 6 - RNA, 67 nt, synthetic construct
  misc_feature 1..67: note = Synthetic oligonucleotide
  source 1..67: mol_type = other RNA
acagcatagcaagttaaaataaggctagtccgttatcaacttgaaaaagtggcaccgagtcggtgct

SEQ ID NO: 7 - RNA, 94 nt, synthetic construct
  misc_feature 1..94: note = Synthetic oligonucleotide
  source 1..94: mol_type = other RNA
gttttcccttttcaaagaaatctcctgggcacctatcttcttaggtgccctcccttgtttaaacctgaccagttaaccggctggttaggttttt

SEQ ID NO: 8 - RNA, 100 nt, synthetic construct
  misc_feature 1..100: note = Synthetic oligonucleotide
  source 1..100: mol_type = other RNA
agtcctcatctccctcaagcgttttagagctagtaatagcaagttaaaataaggctagtccgttatcaacttgaaaaagtggcaccgagtcggtgctttt

SEQ ID NO: 9 - RNA, 113 nt, synthetic construct
  misc_feature 1..113: note = Synthetic oligonucleotide
  source 1..113: mol_type = other RNA
gcagatgtagtgtttccacagtttaagagctatgctggaaacagcatagcaagtttaaataaggctagtccgttatcaacttgaaaaagtggcaccgagtcggtgcttttttt

SEQ ID NO: 10 - RNA, 50 nt, synthetic construct
  misc_feature 1..50: note = Synthetic oligonucleotide
  misc_feature 1..50: note = modified base - um
  source 1..50: mol_type = other RNA
tttttttttttttttttttttttttttttttttttttttttttttttttt